European Patent Application EP 4 541 893 A1, published April 23, 2025. Title: SIRNA MOLECULE FOR REGULATING PCSK9 GENE ACTIVITY. Applicant: RONA BIOSCIENCE, LIMITED. The sequence listing filed with the application follows.

SEQUENCE LISTING (440 sequences)

SEQ ID NO: 1 - RNA, 19 nt, synthetic construct
  misc_feature 1..19: note = sense strand
  source 1..19: mol_type = other RNA
cctacgtggtggtgctgaa

SEQ ID NO: 2 - RNA, 19 nt, synthetic construct
  misc_feature 1..19: note = sense strand
  source 1..19: mol_type = other RNA
ggtggaggtgtatctccta

SEQ ID NO: 3 - RNA, 19 nt, synthetic construct
  misc_feature 1..19: note = sense strand
  source 1..19: mol_type = other RNA
gggtcatggtcaccgactt

SEQ ID NO: 4 - RNA, 19 nt, synthetic construct
  misc_feature 1..19: note = sense strand
  source 1..19: mol_type = other RNA
cctggagtttattcggaaa

SEQ ID NO: 5 - RNA, 19 nt, synthetic construct
  misc_feature 1..19: note = sense strand
  source 1..19: mol_type = other RNA
gcacctgctttgtgtcaca

SEQ ID NO: 6 - RNA, 19 nt, synthetic construct
  misc_feature 1..19: note = sense strand
  source 1..19: mol_type = other RNA
ccaaagatgtcatcaatga

SEQ ID NO: 7 - RNA, 19 nt, synthetic construct
  misc_feature 1..19: note = sense strand
  source 1..19: mol_type = other RNA
gctgttttgcaggactgta

SEQ ID NO: 8 - RNA, 19 nt, synthetic construct
  misc_feature 1..19: note = sense strand
  source 1..19: mol_type = other RNA
ggtctggaatgcaaagtca

SEQ ID NO: 9 - RNA, 19 nt, synthetic construct
  misc_feature 1..19: note = sense strand
  source 1..19: mol_type = other RNA
ggctggggctgagctttaa

SEQ ID NO: 10 - RNA, 19 nt, synthetic construct
  misc_feature 1..19: note = sense strand
  source 1..19: mol_type = other RNA
gcaggaactgagccagaaa

SEQ ID NO: 11 - RNA, 19 nt, synthetic construct
  misc_feature 1..19: note = sense strand
  source 1..19: mol_type = other RNA
ccaagcaagcagacattta

SEQ ID NO: 12 - RNA, 19 nt, synthetic construct
  misc_feature 1..19: note = sense strand
  source 1..19: mol_type = other RNA
ctgtcctctctgttgcctt

SEQ ID NO: 13 - RNA, 19 nt, synthetic construct
  misc_feature 1..19: note = sense strand
  source 1..19: mol_type = other RNA
tgtcctctctgttgccttt

SEQ ID NO: 14 - RNA, 19 nt, synthetic construct
  misc_feature 1..19: note = sense strand
  source 1..19: mol_type = other RNA
gtcctctctgttgcctttt

SEQ ID NO: 15 - RNA, 19 nt, synthetic construct
  misc_feature 1..19: note = sense strand
  source 1..19: mol_type = other RNA
tcctctctgttgccttttt

SEQ ID NO: 16 - RNA, 19 nt, synthetic construct
  misc_feature 1..19: note = sense strand
  source 1..19: mol_type = other RNA
cctctctgttgccttttta

SEQ ID NO: 17 - RNA, 19 nt, synthetic construct
  misc_feature 1..19: note = sense strand
  source 1..19: mol_type = other RNA
ctctctgttgcctttttat

SEQ ID NO: 18 - RNA, 19 nt, synthetic construct
  misc_feature 1..19: note = sense strand
  source 1..19: mol_type = other RNA
tctctgttgcctttttaca

SEQ ID NO: 19 - RNA, 19 nt, synthetic construct
  misc_feature 1..19: note = sense strand
  source 1..19: mol_type = other RNA
ctctgttgcctttttacaa

SEQ ID NO: 20 - RNA, 19 nt, synthetic construct
  misc_feature 1..19: note = sense strand
  source 1..19: mol_type = other RNA
tctgttgcctttttacaga

SEQ ID NO: 21 - RNA, 19 nt, synthetic construct
  misc_feature 1..19: note = sense strand
  source 1..19: mol_type = other RNA
ctgttgcctttttacagca

SEQ ID NO: 22 - RNA, 19 nt, synthetic construct
  misc_feature 1..19: note = sense strand
  source 1..19: mol_type = other RNA
tgttgcctttttacagcca

SEQ ID NO: 23 - RNA, 19 nt, synthetic construct
  misc_feature 1..19: note = sense strand
  source 1..19: mol_type = other RNA
gttgcctttttacagccaa

SEQ ID NO: 24 - RNA, 19 nt, synthetic construct
  misc_feature 1..19: note = sense strand
  source 1..19: mol_type = other RNA
ttgcctttttacagccaaa

SEQ ID NO: 25 - RNA, 19 nt, synthetic construct
  misc_feature 1..19: note = sense strand
  source 1..19: mol_type = other RNA
acttttctagacctgtttt

SEQ ID NO: 26 - RNA, 19 nt, synthetic construct
  misc_feature 1..19: note = sense strand
  source 1..19: mol_type = other RNA
cttttctagacctgtttta

SEQ ID NO: 27 - RNA, 19 nt, synthetic construct
  misc_feature 1..19: note = sense strand
  source 1..19: mol_type = other RNA
ttttctagacctgttttga

SEQ ID NO: 28 - RNA, 19 nt, synthetic construct
  misc_feature 1..19: note = sense strand
  source 1..19: mol_type = other RNA
tttctagacctgttttgct

SEQ ID NO: 29 - RNA, 19 nt, synthetic construct
  misc_feature 1..19: note = sense strand
  source 1..19: mol_type = other RNA
ttctagacctgttttgctt

SEQ ID NO: 30 - RNA, 19 nt, synthetic construct
  misc_feature 1..19: note = sense strand
  source 1..19: mol_type = other RNA
tctagacctgttttgcttt

SEQ ID NO: 31 - RNA, 19 nt, synthetic construct
  misc_feature 1..19: note = sense strand
  source 1..19: mol_type = other RNA
ctagacctgttttgctttt

SEQ ID NO: 32 - RNA, 19 nt, synthetic construct
  misc_feature 1..19: note = sense strand
  source 1..19: mol_type = other RNA
tagacctgttttgctttta

SEQ ID NO: 33 - RNA, 19 nt, synthetic construct
  misc_feature 1..19: note = sense strand
  source 1..19: mol_type = other RNA
agacctgttttgcttttgt

SEQ ID NO: 34 - RNA, 19 nt, synthetic construct
  misc_feature 1..19: note = sense strand
  source 1..19: mol_type = other RNA
gacctgttttgcttttgta

SEQ ID NO: 35 - RNA, 19 nt, synthetic construct
  misc_feature 1..19: note = sense strand
  source 1..19: mol_type = other RNA
acctgttttgcttttgtaa

SEQ ID NO: 36 - RNA, 19 nt, synthetic construct
  misc_feature 1..19: note = sense strand
  source 1..19: mol_type = other RNA
cctgttttgcttttgtaaa

SEQ ID NO: 37 - RNA, 19 nt, synthetic construct
  misc_feature 1..19: note = sense strand
  source 1..19: mol_type = other RNA
ctgttttgcttttgtaact

SEQ ID NO: 38 - RNA, 19 nt, synthetic construct
  misc_feature 1..19: note = sense strand
  source 1..19: mol_type = other RNA
tgttttgcttttgtaactt

SEQ ID NO: 39 - RNA, 19 nt, synthetic construct
  misc_feature 1..19: note = sense strand
  source 1..19: mol_type = other RNA
gttttgcttttgtaactta

SEQ ID NO: 40 - RNA, 19 nt, synthetic construct
  misc_feature 1..19: note = sense strand
  source 1..19: mol_type = other RNA
ttttgcttttgtaacttga

SEQ ID NO: 41 - RNA, 19 nt, synthetic construct
  misc_feature 1..19: note = sense strand
  source 1..19: mol_type = other RNA
tttgcttttgtaacttgaa

SEQ ID NO: 42 - RNA, 19 nt, synthetic construct
  misc_feature 1..19: note = sense strand
  source 1..19: mol_type = other RNA
ttgcttttgtaacttgaaa

SEQ ID NO: 43 - RNA, 19 nt, synthetic construct
  misc_feature 1..19: note = sense strand
  source 1..19: mol_type = other RNA
tgcttttgtaacttgaaga

SEQ ID NO: 44 - RNA, 19 nt, synthetic construct
  misc_feature 1..19: note = sense strand
  source 1..19: mol_type = other RNA
gcttttgtaacttgaagat

SEQ ID NO: 45 - RNA, 19 nt, synthetic construct
  misc_feature 1..19: note = sense strand
  source 1..19: mol_type = other RNA
cttttgtaacttgaagata

SEQ ID NO: 46 - RNA, 19 nt, synthetic construct
  misc_feature 1..19: note = sense strand
  source 1..19: mol_type = other RNA
ttttgtaacttgaagatat

SEQ ID NO: 47 - RNA, 19 nt, synthetic construct
  misc_feature 1..19: note = sense strand
  source 1..19: mol_type = other RNA
tttgtaacttgaagatatt

SEQ ID NO: 48 - RNA, 19 nt, synthetic construct
  misc_feature 1..19: note = sense strand
  source 1..19: mol_type = other RNA
ttgtaacttgaagatattt

SEQ ID NO: 49 - RNA, 19 nt, synthetic construct
  misc_feature 1..19: note = sense strand
  source 1..19: mol_type = other RNA
tgtaacttgaagatattta

SEQ ID NO: 50 - RNA, 19 nt, synthetic construct
  misc_feature 1..19: note = sense strand
  source 1..19: mol_type = other RNA
gtaacttgaagatatttat

SEQ ID NO: 51 - RNA, 19 nt, synthetic construct
  misc_feature 1..19: note = sense strand
  source 1..19: mol_type = other RNA
taacttgaagatatttatt

SEQ ID NO: 52 - RNA, 19 nt, synthetic construct
  misc_feature 1..19: note = sense strand
  source 1..19: mol_type = other RNA
aacttgaagatatttatta

SEQ ID NO: 53 - RNA, 19 nt, synthetic construct
  misc_feature 1..19: note = sense strand
  source 1..19: mol_type = other RNA
acttgaagatatttattct

SEQ ID NO: 54 - RNA, 19 nt, synthetic construct
  misc_feature 1..19: note = sense strand
  source 1..19: mol_type = other RNA
cttgaagatatttattcta

SEQ ID NO: 55 - RNA, 19 nt, synthetic construct
  misc_feature 1..19: note = sense strand
  source 1..19: mol_type = other RNA
ttgaagatatttattctga

SEQ ID NO: 56 - RNA, 19 nt, synthetic construct
  misc_feature 1..19: note = sense strand
  source 1..19: mol_type = other RNA
tgaagatatttattctgga

SEQ ID NO: 57 - RNA, 19 nt, synthetic construct
  misc_feature 1..19: note = sense strand
  source 1..19: mol_type = other RNA
gaagatatttattctgggt

SEQ ID NO: 58 - RNA, 19 nt, synthetic construct
  misc_feature 1..19: note = sense strand
  source 1..19: mol_type = other RNA
aagatatttattctgggtt

SEQ ID NO: 59 - RNA, 19 nt, synthetic construct
  misc_feature 1..19: note = sense strand
  source 1..19: mol_type = other RNA
agatatttattctgggttt

SEQ ID NO: 60 - RNA, 19 nt, synthetic construct
  misc_feature 1..19: note = sense strand
  source 1..19: mol_type = other RNA
gatatttattctgggtttt

SEQ ID NO: 61 - RNA, 19 nt, synthetic construct
  misc_feature 1..19: note = sense strand
  source 1..19: mol_type = other RNA
atatttattctgggtttta

SEQ ID NO: 62 - RNA, 19 nt, synthetic construct
  misc_feature 1..19: note = sense strand
  source 1..19: mol_type = other RNA
tatttattctgggttttgt

SEQ ID NO: 63 - RNA, 19 nt, synthetic construct
  misc_feature 1..19: note = sense strand
  source 1..19: mol_type = other RNA
atttattctgggttttgta

SEQ ID NO: 64 - RNA, 19 nt, synthetic construct
  misc_feature 1..19: note = sense strand
  source 1..19: mol_type = other RNA
tttattctgggttttgtaa

SEQ ID NO: 65 - RNA, 19 nt, synthetic construct
  misc_feature 1..19: note = sense strand
  source 1..19: mol_type = other RNA
ttattctgggttttgtaga

SEQ ID NO: 66 - RNA, 19 nt, synthetic construct
  misc_feature 1..19: note = sense strand
  source 1..19: mol_type = other RNA
tattctgggttttgtagca

SEQ ID NO: 67 - RNA, 19 nt, synthetic construct
  misc_feature 1..19: note = sense strand
  source 1..19: mol_type = other RNA
attctgggttttgtagcat

SEQ ID NO: 68 - RNA, 19 nt, synthetic construct
  misc_feature 1..19: note = sense strand
  source 1..19: mol_type = other RNA
ttctgggttttgtagcatt

SEQ ID NO: 69 - RNA, 19 nt, synthetic construct
  misc_feature 1..19: note = sense strand
  source 1..19: mol_type = other RNA
tctgggttttgtagcattt

SEQ ID NO: 70 - RNA, 19 nt, synthetic construct
  misc_feature 1..19: note = sense strand
  source 1..19: mol_type = other RNA
ctgggttttgtagcatttt

SEQ ID NO: 71 - RNA, 19 nt, synthetic construct
  misc_feature 1..19: note = sense strand
  source 1..19: mol_type = other RNA
tgggttttgtagcattttt

SEQ ID NO: 72 - RNA, 19 nt, synthetic construct
  misc_feature 1..19: note = sense strand
  source 1..19: mol_type = other RNA
gggttttgtagcattttta

SEQ ID NO: 73 - RNA, 19 nt, synthetic construct
  misc_feature 1..19: note = sense strand
  source 1..19: mol_type = other RNA
ggttttgtagcatttttat

SEQ ID NO: 74 - RNA, 19 nt, synthetic construct
  misc_feature 1..19: note = sense strand
  source 1..19: mol_type = other RNA
gttttgtagcatttttatt

SEQ ID NO: 75 - RNA, 19 nt, synthetic construct
  misc_feature 1..19: note = sense strand
  source 1..19: mol_type = other RNA
ttttgtagcatttttatta

SEQ ID NO: 76 - RNA, 19 nt, synthetic construct
  misc_feature 1..19: note = sense strand
  source 1..19: mol_type = other RNA
tttgtagcatttttattaa

SEQ ID NO: 77 - RNA, 19 nt, synthetic construct
  misc_feature 1..19: note = sense strand
  source 1..19: mol_type = other RNA
ttgtagcatttttattaat

SEQ ID NO: 78 - RNA, 19 nt, synthetic construct
  misc_feature 1..19: note = sense strand
  source 1..19: mol_type = other RNA
tgtagcatttttattaata

SEQ ID NO: 79 - RNA, 19 nt, synthetic construct
  misc_feature 1..19: note = sense strand
  source 1..19: mol_type = other RNA
gtagcatttttattaatat

SEQ ID NO: 80 - RNA, 19 nt, synthetic construct
  misc_feature 1..19: note = sense strand
  source 1..19: mol_type = other RNA
tagcatttttattaatata

SEQ ID NO: 81 - RNA, 19 nt, synthetic construct
  misc_feature 1..19: note = sense strand
  source 1..19: mol_type = other RNA
agcatttttattaatatga

SEQ ID NO: 82 - RNA, 19 nt, synthetic construct
  misc_feature 1..19: note = sense strand
  source 1..19: mol_type = other RNA
ggtgactttttaaaataaa

SEQ ID NO: 83 - RNA, 19 nt, synthetic construct
  misc_feature 1..19: note = sense strand
  source 1..19: mol_type = other RNA
gtgactttttaaaataaaa

SEQ ID NO: 84 - RNA, 19 nt, synthetic construct
  misc_feature 1..19: note = sense strand
  source 1..19: mol_type = other RNA
tgactttttaaaataaaaa

SEQ ID NO: 85 - RNA, 19 nt, synthetic construct
  misc_feature 1..19: note = sense strand
  source 1..19: mol_type = other RNA
gactttttaaaataaaaat

SEQ ID NO: 86 - RNA, 19 nt, synthetic construct
  misc_feature 1..19: note = sense strand
  source 1..19: mol_type = other RNA
actttttaaaataaaaaca

SEQ ID NO: 87 - RNA, 19 nt, synthetic construct
  misc_feature 1..19: note = sense strand
  source 1..19: mol_type = other RNA
ctttttaaaataaaaacaa

SEQ ID NO: 88 - RNA, 19 nt, synthetic construct
  misc_feature 1..19: note = sense strand
  source 1..19: mol_type = other RNA
tttttaaaataaaaacaaa

SEQ ID NO: 89 - RNA, 19 nt, synthetic construct
  misc_feature 1..19: note = sense strand
  source 1..19: mol_type = other RNA
ttttaaaataaaaacaaat

SEQ ID NO: 90 - RNA, 19 nt, synthetic construct
  misc_feature 1..19: note = sense strand
  source 1..19: mol_type = other RNA
tttaaaataaaaacaaaca

SEQ ID NO: 91 - RNA, 21 nt, synthetic construct
  source 1..21: mol_type = other RNA
  misc_feature 1..21: note = sense strand
  misc_feature 11: note = T is dT
ctagacctgttttgcttttgt

SEQ ID NO: 92 - RNA, 19 nt, synthetic construct
  misc_feature 1..19: note = sense strand
  source 1..19: mol_type = other RNA
tgttttgcttttgtaactt

SEQ ID NO: 93 - RNA, 19 nt, synthetic construct
  misc_feature 1..19: note = sense strand
  source 1..19: mol_type = other RNA
gttttgcttttgtaactta

SEQ ID NO: 94 - RNA, 19 nt, synthetic construct
  misc_feature 1..19: note = sense strand
  source 1..19: mol_type = other RNA
ttttgcttttgtaacttga

SEQ ID NO: 95 - RNA, 19 nt, synthetic construct
  misc_feature 1..19: note = sense strand
  source 1..19: mol_type = other RNA
tgcttttgtaacttgaaga

SEQ ID NO: 96 - RNA, 19 nt, synthetic construct
  misc_feature 1..19: note = sense strand
  source 1..19: mol_type = other RNA
gcttttgtaacttgaagat

SEQ ID NO: 97 - RNA, 19 nt, synthetic construct
  misc_feature 1..19: note = sense strand
  source 1..19: mol_type = other RNA
cttttgtaacttgaagata

SEQ ID NO: 98 - RNA, 19 nt, synthetic construct
  misc_feature 1..19: note = sense strand
  source 1..19: mol_type = other RNA
ttttgtaacttgaagatat

SEQ ID NO: 99 - RNA, 21 nt, synthetic construct
  source 1..21: mol_type = other RNA
  misc_feature 1..21: note = sense strand
  misc_feature 11: note = T is dT
ctagacctgttttgcttttgt

SEQ ID NO: 100 - RNA, 21 nt, synthetic construct
  source 1..21: mol_type = other RNA
  misc_feature 1..21: note = sense strand
  misc_feature 11: note = T is dT
ctagacctgttttgcttttgt

SEQ ID NO: 101 - RNA, 19 nt, synthetic construct
  misc_feature 1..19: note = sense strand
  source 1..19: mol_type = other RNA
gttttgcttttgtaactta

SEQ ID NO: 102 - RNA, 19 nt, synthetic construct
  misc_feature 1..19: note = sense strand
  source 1..19: mol_type = other RNA
gttttgcttttgtaactta

SEQ ID NO: 103 - RNA, 19 nt, synthetic construct
  misc_feature 1..19: note = sense strand
  source 1..19: mol_type = other RNA
tgttttgcttttgtaactt

SEQ ID NO: 104 - RNA, 19 nt, synthetic construct
  misc_feature 1..19: note = sense strand
  source 1..19: mol_type = other RNA
tgcttttgtaacttgaaga

SEQ ID NO: 105 - RNA, 21 nt, synthetic construct
  misc_feature 1..21: note = antisense strand
  source 1..21: mol_type = other RNA
ttcagcaccaccacgtaggtg

SEQ ID NO: 106 - RNA, 21 nt, synthetic construct
  misc_feature 1..21: note = antisense strand
  source 1..21: mol_type = other RNA
taggagatacacctccaccag

SEQ ID NO: 107 - RNA, 21 nt, synthetic construct
  misc_feature 1..21: note = antisense strand
  source 1..21: mol_type = other RNA
aagtcggtgaccatgaccctg

SEQ ID NO: 108 - RNA, 21 nt, synthetic construct
  misc_feature 1..21: note = antisense strand
  source 1..21: mol_type = other RNA
tttccgaataaactccaggcc

SEQ ID NO: 109 - RNA, 21 nt, synthetic construct
  misc_feature 1..21: note = antisense strand
  source 1..21: mol_type = other RNA
tgtgacacaaagcaggtgctg

SEQ ID NO: 110 - RNA, 21 nt, synthetic construct
  misc_feature 1..21: note = antisense strand
  source 1..21: mol_type = other RNA
tcattgatgacatctttggca

SEQ ID NO: 111 - RNA, 21 nt, synthetic construct
  misc_feature 1..21: note = antisense strand
  source 1..21: mol_type = other RNA
tacagtcctgcaaaacagctg

SEQ ID NO: 112 - RNA, 21 nt, synthetic construct
  misc_feature 1..21: note = antisense strand
  source 1..21: mol_type = other RNA
tgactttgcattccagacctg

SEQ ID NO: 113 - RNA, 21 nt, synthetic construct
  misc_feature 1..21: note = antisense strand
  source 1..21: mol_type = other RNA
ttaaagctcagccccagccct

SEQ ID NO: 114 - RNA, 21 nt, synthetic construct
  misc_feature 1..21: note = antisense strand
  source 1..21: mol_type = other RNA
tttctggctcagttcctgctg

SEQ ID NO: 115 - RNA, 21 nt, synthetic construct
  misc_feature 1..21: note = antisense strand
  source 1..21: mol_type = other RNA
taaatgtctgcttgcttgggt

SEQ ID NO: 116 - RNA, 21 nt, synthetic construct
  misc_feature 1..21: note = antisense strand
  source 1..21: mol_type = other RNA
aaggcaacagagaggacagac

SEQ ID NO: 117 - RNA, 21 nt, synthetic construct
  misc_feature 1..21: note = antisense strand
  source 1..21: mol_type = other RNA
aaaggcaacagagaggacaga

SEQ ID NO: 118 - RNA, 21 nt, synthetic construct
  misc_feature 1..21: note = antisense strand
  source 1..21: mol_type = other RNA
aaaaggcaacagagaggacag

SEQ ID NO: 119 - RNA, 21 nt, synthetic construct
  misc_feature 1..21: note = antisense strand
  source 1..21: mol_type = other RNA
aaaaaggcaacagagaggaca

SEQ ID NO: 120 - RNA, 21 nt, synthetic construct
  misc_feature 1..21: note = antisense strand
  source 1..21: mol_type = other RNA
taaaaaggcaacagagaggac

SEQ ID NO: 121 - RNA, 21 nt, synthetic construct
  misc_feature 1..21: note = antisense strand
  source 1..21: mol_type = other RNA
ataaaaaggcaacagagagga

SEQ ID NO: 122 - RNA, 21 nt, synthetic construct
  misc_feature 1..21: note = antisense strand
  source 1..21: mol_type = other RNA
tgtaaaaaggcaacagagagg

SEQ ID NO: 123 - RNA, 21 nt, synthetic construct
  misc_feature 1..21: note = antisense strand
  source 1..21: mol_type = other RNA
ttgtaaaaaggcaacagagag

SEQ ID NO: 124 - RNA, 21 nt, synthetic construct
  misc_feature 1..21: note = antisense strand
  source 1..21: mol_type = other RNA
tctgtaaaaaggcaacagaga

SEQ ID NO: 125 - RNA, 21 nt, synthetic construct
  misc_feature 1..21: note = antisense strand
  source 1..21: mol_type = other RNA
tgctgtaaaaaggcaacagag

SEQ ID NO: 126 - RNA, 21 nt, synthetic construct
  misc_feature 1..21: note = antisense strand
  source 1..21: mol_type = other RNA
tggctgtaaaaaggcaacaga

SEQ ID NO: 127 - RNA, 21 nt, synthetic construct
  misc_feature 1..21: note = antisense strand
  source 1..21: mol_type = other RNA
ttggctgtaaaaaggcaacag

SEQ ID NO: 128 - RNA, 21 nt, synthetic construct
  misc_feature 1..21: note = antisense strand
  source 1..21: mol_type = other RNA
tttggctgtaaaaaggcaaca

SEQ ID NO: 129 - RNA, 21 nt, synthetic construct
  misc_feature 1..21: note = antisense strand
  source 1..21: mol_type = other RNA
aaaacaggtctagaaaagttg

SEQ ID NO: 130 - RNA, 21 nt, synthetic construct
  misc_feature 1..21: note = antisense strand
  source 1..21: mol_type = other RNA
taaaacaggtctagaaaagtt

SEQ ID NO: 131 - RNA, 21 nt, synthetic construct
  misc_feature 1..21: note = antisense strand
  source 1..21: mol_type = other RNA
tcaaaacaggtctagaaaagt

SEQ ID NO: 132 - RNA, 21 nt, synthetic construct
  misc_feature 1..21: note = antisense strand
  source 1..21: mol_type = other RNA
agcaaaacaggtctagaaaag

SEQ ID NO: 133 - RNA, 21 nt, synthetic construct
  misc_feature 1..21: note = antisense strand
  source 1..21: mol_type = other RNA
aagcaaaacaggtctagaaaa

SEQ ID NO: 134 - RNA, 21 nt, synthetic construct
  misc_feature 1..21: note = antisense strand
  source 1..21: mol_type = other RNA
aaagcaaaacaggtctagaaa

SEQ ID NO: 135 - RNA, 21 nt, synthetic construct
  misc_feature 1..21: note = antisense strand
  source 1..21: mol_type = other RNA
aaaagcaaaacaggtctagaa

SEQ ID NO: 136 - RNA, 21 nt, synthetic construct
  misc_feature 1..21: note = antisense strand
  source 1..21: mol_type = other RNA
taaaagcaaaacaggtctaga

SEQ ID NO: 137 - RNA, 21 nt, synthetic construct
  misc_feature 1..21: note = antisense strand
  source 1..21: mol_type = other RNA
acaaaagcaaaacaggtctag

SEQ ID NO: 138 - RNA, 21 nt, synthetic construct
  misc_feature 1..21: note = antisense strand
  source 1..21: mol_type = other RNA
tacaaaagcaaaacaggtcta

SEQ ID NO: 139 - RNA, 21 nt, synthetic construct
  misc_feature 1..21: note = antisense strand
  source 1..21: mol_type = other RNA
ttacaaaagcaaaacaggtct

SEQ ID NO: 140 - RNA, 21 nt, synthetic construct
  misc_feature 1..21: note = antisense strand
  source 1..21: mol_type = other RNA
tttacaaaagcaaaacaggtc

SEQ ID NO: 141 - RNA, 21 nt, synthetic construct
  misc_feature 1..21: note = antisense strand
  source 1..21: mol_type = other RNA
agttacaaaagcaaaacaggt

SEQ ID NO: 142 - RNA, 21 nt, synthetic construct
  misc_feature 1..21: note = antisense strand
  source 1..21: mol_type = other RNA
aagttacaaaagcaaaacagg

SEQ ID NO: 143 - RNA, 21 nt, synthetic construct
  misc_feature 1..21: note = antisense strand
  source 1..21: mol_type = other RNA
taagttacaaaagcaaaacag

SEQ ID NO: 144 - RNA, 21 nt, synthetic construct
  misc_feature 1..21: note = antisense strand
  source 1..21: mol_type = other RNA
tcaagttacaaaagcaaaaca

SEQ ID NO: 145 - RNA, 21 nt, synthetic construct
  misc_feature 1..21: note = antisense strand
  source 1..21: mol_type = other RNA
ttcaagttacaaaagcaaaac

SEQ ID NO: 146 - RNA, 21 nt, synthetic construct
  misc_feature 1..21: note = antisense strand
  source 1..21: mol_type = other RNA
tttcaagttacaaaagcaaaa

SEQ ID NO: 147 - RNA, 21 nt, synthetic construct
  misc_feature 1..21: note = antisense strand
  source 1..21: mol_type = other RNA
tcttcaagttacaaaagcaaa

SEQ ID NO: 148 - RNA, 21 nt, synthetic construct
  misc_feature 1..21: note = antisense strand
  source 1..21: mol_type = other RNA
atcttcaagttacaaaagcaa

SEQ ID NO: 149 - RNA, 21 nt, synthetic construct
  misc_feature 1..21: note = antisense strand
  source 1..21: mol_type = other RNA
tatcttcaagttacaaaagca

SEQ ID NO: 150 - RNA, 21 nt, synthetic construct
  misc_feature 1..21: note = antisense strand
  source 1..21: mol_type = other RNA
atatcttcaagttacaaaagc

SEQ ID NO: 151 - RNA, 21 nt, synthetic construct
  misc_feature 1..21: note = antisense strand
  source 1..21: mol_type = other RNA
aatatcttcaagttacaaaag

SEQ ID NO: 152 - RNA, 21 nt, synthetic construct
  misc_feature 1..21: note = antisense strand
  source 1..21: mol_type = other RNA
aaatatcttcaagttacaaaa

SEQ ID NO: 153 - RNA, 21 nt, synthetic construct
  misc_feature 1..21: note = antisense strand
  source 1..21: mol_type = other RNA
taaatatcttcaagttacaaa

SEQ ID NO: 154 - RNA, 21 nt, synthetic construct
  misc_feature 1..21: note = antisense strand
  source 1..21: mol_type = other RNA
ataaatatcttcaagttacaa

SEQ ID NO: 155 - RNA, 21 nt, synthetic construct
  misc_feature 1..21: note = antisense strand
  source 1..21: mol_type = other RNA
aataaatatcttcaagttaca

SEQ ID NO: 156 - RNA, 21 nt, synthetic construct
  misc_feature 1..21: note = antisense strand
  source 1..21: mol_type = other RNA
taataaatatcttcaagttac

SEQ ID NO: 157 - RNA, 21 nt, synthetic construct
  misc_feature 1..21: note = antisense strand
  source 1..21: mol_type = other RNA
agaataaatatcttcaagtta

SEQ ID NO: 158 - RNA, 21 nt, synthetic construct
  misc_feature 1..21: note = antisense strand
  source 1..21: mol_type = other RNA
tagaataaatatcttcaagtt

SEQ ID NO: 159 - RNA, 21 nt, synthetic construct
  misc_feature 1..21: note = antisense strand
  source 1..21: mol_type = other RNA
tcagaataaatatcttcaagt

SEQ ID NO: 160 - RNA, 21 nt, synthetic construct
  misc_feature 1..21: note = antisense strand
  source 1..21: mol_type = other RNA
tccagaataaatatcttcaag

SEQ ID NO: 161 - RNA, 21 nt, synthetic construct
  misc_feature 1..21: note = antisense strand
  source 1..21: mol_type = other RNA
acccagaataaatatcttcaa

SEQ ID NO: 162 - RNA, 21 nt, synthetic construct
  misc_feature 1..21: note = antisense strand
  source 1..21: mol_type = other RNA
aacccagaataaatatcttca

SEQ ID NO: 163 - RNA, 21 nt, synthetic construct
  misc_feature 1..21: note = antisense strand
  source 1..21: mol_type = other RNA
aaacccagaataaatatcttc

SEQ ID NO: 164 - RNA, 21 nt, synthetic construct
  misc_feature 1..21: note = antisense strand
  source 1..21: mol_type = other RNA
aaaacccagaataaatatctt

SEQ ID NO: 165 - RNA, 21 nt, synthetic construct
  misc_feature 1..21: note = antisense strand
  source 1..21: mol_type = other RNA
taaaacccagaataaatatct

SEQ ID NO: 166 - RNA, 21 nt, synthetic construct
  misc_feature 1..21: note = antisense strand
  source 1..21: mol_type = other RNA
acaaaacccagaataaatatc

SEQ ID NO: 167 - RNA, 21 nt, synthetic construct
  misc_feature 1..21: note = antisense strand
  source 1..21: mol_type = other RNA
tacaaaacccagaataaatat

SEQ ID NO: 168 - RNA, 21 nt, synthetic construct
  misc_feature 1..21: note = antisense strand
  source 1..21: mol_type = other RNA
ttacaaaacccagaataaata

SEQ ID NO: 169 - RNA, 21 nt, synthetic construct
  misc_feature 1..21: note = antisense strand
  source 1..21: mol_type = other RNA
tctacaaaacccagaataaat

SEQ ID NO: 170 - RNA, 21 nt, synthetic construct
  misc_feature 1..21: note = antisense strand
  source 1..21: mol_type = other RNA
tgctacaaaacccagaataaa

SEQ ID NO: 171 - RNA, 21 nt, synthetic construct
  misc_feature 1..21: note = antisense strand
  source 1..21: mol_type = other RNA
atgctacaaaacccagaataa

SEQ ID NO: 172 - RNA, 21 nt, synthetic construct
  misc_feature 1..21: note = antisense strand
  source 1..21: mol_type = other RNA
aatgctacaaaacccagaata

SEQ ID NO: 173 - RNA, 21 nt, synthetic construct
  misc_feature 1..21: note = antisense strand
  source 1..21: mol_type = other RNA
aaatgctacaaaacccagaat

SEQ ID NO: 174 - RNA, 21 nt, synthetic construct
  misc_feature 1..21: note = antisense strand
  source 1..21: mol_type = other RNA
aaaatgctacaaaacccagaa

SEQ ID NO: 175 - RNA, 21 nt, synthetic construct
  misc_feature 1..21: note = antisense strand
  source 1..21: mol_type = other RNA
aaaaatgctacaaaacccaga

SEQ ID NO: 176 - RNA, 21 nt, synthetic construct
  misc_feature 1..21: note = antisense strand
  source 1..21: mol_type = other RNA
taaaaatgctacaaaacccag

SEQ ID NO: 177 - RNA, 21 nt, synthetic construct
  misc_feature 1..21: note = antisense strand
  source 1..21: mol_type = other RNA
ataaaaatgctacaaaaccca

SEQ ID NO: 178 - RNA, 21 nt, synthetic construct
  misc_feature 1..21: note = antisense strand
  source 1..21: mol_type = other RNA
aataaaaatgctacaaaaccc

SEQ ID NO: 179 - RNA, 21 nt, synthetic construct
  misc_feature 1..21: note = antisense strand
  source 1..21: mol_type = other RNA
taataaaaatgctacaaaacc

SEQ ID NO: 180 - RNA, 21 nt, synthetic construct
  misc_feature 1..21: note = antisense strand
  source 1..21: mol_type = other RNA
ttaataaaaatgctacaaaac

SEQ ID NO: 181 - RNA, 21 nt, synthetic construct
  misc_feature 1..21: note = antisense strand
  source 1..21: mol_type = other RNA
attaataaaaatgctacaaaa

SEQ ID NO: 182 - RNA, 21 nt, synthetic construct
  misc_feature 1..21: note = antisense strand
  source 1..21: mol_type = other RNA
tattaataaaaatgctacaaa

SEQ ID NO: 183 - RNA, 21 nt, synthetic construct
  misc_feature 1..21: note = antisense strand
  source 1..21: mol_type = other RNA
atattaataaaaatgctacaa

SEQ ID NO: 184 - RNA, 21 nt, synthetic construct
  misc_feature 1..21: note = antisense strand
  source 1..21: mol_type = other RNA
tatattaataaaaatgctaca

SEQ ID NO: 185 - RNA, 21 nt, synthetic construct
  misc_feature 1..21: note = antisense strand
  source 1..21: mol_type = other RNA
tcatattaataaaaatgctac

SEQ ID NO: 186 - RNA, 21 nt, synthetic construct
  misc_feature 1..21: note = antisense strand
  source 1..21: mol_type = other RNA
tttattttaaaaagtcaccat

SEQ ID NO: 187 - RNA, 21 nt, synthetic construct
  misc_feature 1..21: note = antisense strand
  source 1..21: mol_type = other RNA
ttttattttaaaaagtcacca

SEQ ID NO: 188 - RNA, 21 nt, synthetic construct
  misc_feature 1..21: note = antisense strand
  source 1..21: mol_type = other RNA
tttttattttaaaaagtcacc

SEQ ID NO: 189 - RNA, 21 nt, synthetic construct
  misc_feature 1..21: note = antisense strand
  source 1..21: mol_type = other RNA
atttttattttaaaaagtcac

SEQ ID NO: 190 - RNA, 21 nt, synthetic construct
  misc_feature 1..21: note = antisense strand
  source 1..21: mol_type = other RNA
tgtttttattttaaaaagtca

SEQ ID NO: 191 - RNA, 21 nt, synthetic construct
  misc_feature 1..21: note = antisense strand
  source 1..21: mol_type = other RNA
ttgtttttattttaaaaagtc

SEQ ID NO: 192 - RNA, 21 nt, synthetic construct
  misc_feature 1..21: note = antisense strand
  source 1..21: mol_type = other RNA
tttgtttttattttaaaaagt

SEQ ID NO: 193 - RNA, 21 nt, synthetic construct
  misc_feature 1..21: note = antisense strand
  source 1..21: mol_type = other RNA
atttgtttttattttaaaaag

SEQ ID NO: 194 - RNA, 21 nt, synthetic construct
  misc_feature 1..21: note = antisense strand
  source 1..21: mol_type = other RNA
tgtttgtttttattttaaaaa

SEQ ID NO: 195 - RNA, 23 nt, synthetic construct
  misc_feature 1..23: note = antisense strand
  source 1..23: mol_type = other RNA
acaaaagcaaaacaggtctagaa

SEQ ID NO: 196 - RNA, 21 nt, synthetic construct
  misc_feature 1..21: note = antisense strand
  source 1..21: mol_type = other RNA
aagttacaaaagcaaaacagg

SEQ ID NO: 197 - RNA, 21 nt, synthetic construct
  misc_feature 1..21: note = antisense strand
  source 1..21: mol_type = other RNA
taagttacaaaagcaaaacag

SEQ ID NO: 198 - RNA, 21 nt, synthetic construct
  misc_feature 1..21: note = antisense strand
  source 1..21: mol_type = other RNA
tcaagttacaaaagcaaaaca

SEQ ID NO: 199 - RNA, 21 nt, synthetic construct
  misc_feature 1..21: note = antisense strand
  source 1..21: mol_type = other RNA
tcttcaagttacaaaagcaaa

SEQ ID NO: 200 - RNA, 21 nt, synthetic construct
  misc_feature 1..21: note = antisense strand
  source 1..21: mol_type = other RNA
atcttcaagttacaaaagcaa

SEQ ID NO: 201 - RNA, 21 nt, synthetic construct
  misc_feature 1..21: note = antisense strand
  source 1..21: mol_type = other RNA
tatcttcaagttacaaaagca

SEQ ID NO: 202 - RNA, 21 nt, synthetic construct
  misc_feature 1..21: note = antisense strand
  source 1..21: mol_type = other RNA
atatcttcaagttacaaaagc

SEQ ID NO: 203 - RNA, 23 nt, synthetic construct
  misc_feature 1..23: note = antisense strand
  source 1..23: mol_type = other RNA
acaaaagcaaaacaggtctagaa

SEQ ID NO: 204 - RNA, 23 nt, synthetic construct
  misc_feature 1..23: note = antisense strand
  source 1..23: mol_type = other RNA
acaaaagcaaaacaggtctagaa

SEQ ID NO: 205 - RNA, 21 nt, synthetic construct
  misc_feature 1..21: note = antisense strand
  source 1..21: mol_type = other RNA
taagttacaaaagcaaaacag

SEQ ID NO: 206 - RNA, 21 nt, synthetic construct
  misc_feature 1..21: note = antisense strand
  source 1..21: mol_type = other RNA
taagttacaaaagcaaaacag

SEQ ID NO: 207 - RNA, 21 nt, synthetic construct
  misc_feature 1..21: note = antisense strand
  source 1..21: mol_type = other RNA
aagttacaaaagcaaaacagg

SEQ ID NO: 208 - RNA, 21 nt, synthetic construct
  misc_feature 1..21: note = antisense strand
  source 1..21: mol_type = other RNA
tcttcaagttacaaaagcaaa

SEQ ID NO: 209 - RNA, 19 nt, synthetic construct
  misc_feature 1..19: note = SR004482S
  source 1..19: mol_type = other RNA
cctacgtggtggtgctgaa

SEQ ID NO: 210 - RNA, 19 nt, synthetic construct
  misc_feature 1..19: note = SR004483S
  source 1..19: mol_type = other RNA
ggtggaggtgtatctccta

SEQ ID NO: 211 - RNA, 19 nt, synthetic construct
  misc_feature 1..19: note = SR004484S
  source 1..19: mol_type = other RNA
gggtcatggtcaccgactt

SEQ ID NO: 212 - RNA, 19 nt, synthetic construct
  misc_feature 1..19: note = SR004485S
  source 1..19: mol_type = other RNA
cctggagtttattcggaaa

SEQ ID NO: 213 - RNA, 19 nt, synthetic construct
  misc_feature 1..19: note = SR004486S
  source 1..19: mol_type = other RNA
gcacctgctttgtgtcaca

SEQ ID NO: 214 - RNA, 19 nt, synthetic construct
  misc_feature 1..19: note = SR004487S
  source 1..19: mol_type = other RNA
ccaaagatgtcatcaatga

SEQ ID NO: 215 - RNA, 19 nt, synthetic construct
  misc_feature 1..19: note = SR004488S
  source 1..19: mol_type = other RNA
gctgttttgcaggactgta

SEQ ID NO: 216 - RNA, 19 nt, synthetic construct
  misc_feature 1..19: note = SR004489S
  source 1..19: mol_type = other RNA
ggtctggaatgcaaagtca

SEQ ID NO: 217 - RNA, 19 nt, synthetic construct
  misc_feature 1..19: note = SR004490S
  source 1..19: mol_type = other RNA
ggctggggctgagctttaa

SEQ ID NO: 218 - RNA, 19 nt, synthetic construct
  misc_feature 1..19: note = SR004491S
  source 1..19: mol_type = other RNA
gcaggaactgagccagaaa

SEQ ID NO: 219 - RNA, 19 nt, synthetic construct
  misc_feature 1..19: note = SR004492S
  source 1..19: mol_type = other RNA
ccaagcaagcagacattta

SEQ ID NO: 220 - RNA, 19 nt, synthetic construct
  misc_feature 1..19: note = SR004493S
  source 1..19: mol_type = other RNA
ctgtcctctctgttgcctt

SEQ ID NO: 221 - RNA, 19 nt, synthetic construct
  misc_feature 1..19: note = SR004494S
  source 1..19: mol_type = other RNA
tgtcctctctgttgccttt

SEQ ID NO: 222 - RNA, 19 nt, synthetic construct
  misc_feature 1..19: note = SR004495S
  source 1..19: mol_type = other RNA
gtcctctctgttgcctttt

SEQ ID NO: 223 - RNA, 19 nt, synthetic construct
  misc_feature 1..19: note = SR004496S
  source 1..19: mol_type = other RNA
tcctctctgttgccttttt

SEQ ID NO: 224 - RNA, 19 nt, synthetic construct
  misc_feature 1..19: note = SR004497S
  source 1..19: mol_type = other RNA
cctctctgttgccttttta

SEQ ID NO: 225 - RNA, 19 nt, synthetic construct
  misc_feature 1..19: note = SR004498S
  source 1..19: mol_type = other RNA
ctctctgttgcctttttat

SEQ ID NO: 226 - RNA, 19 nt, synthetic construct
  misc_feature 1..19: note = SR004499S
  source 1..19: mol_type = other RNA
tctctgttgcctttttaca

SEQ ID NO: 227 - RNA, 19 nt, synthetic construct
  misc_feature 1..19: note = SR004500S
  source 1..19: mol_type = other RNA
ctctgttgcctttttacaa

SEQ ID NO: 228 - RNA, 19 nt, synthetic construct
  misc_feature 1..19: note = SR004501S
  source 1..19: mol_type = other RNA
tctgttgcctttttacaga

SEQ ID NO: 229 - RNA, 19 nt, synthetic construct
  misc_feature 1..19: note = SR004502S
  source 1..19: mol_type = other RNA
ctgttgcctttttacagca

SEQ ID NO: 230 - RNA, 19 nt, synthetic construct
  misc_feature 1..19: note = SR004503S
  source 1..19: mol_type = other RNA
tgttgcctttttacagcca

SEQ ID NO: 231 - RNA, 19 nt, synthetic construct
  misc_feature 1..19: note = SR004504S
  source 1..19: mol_type = other RNA
gttgcctttttacagccaa

SEQ ID NO: 232 - RNA, 19 nt, synthetic construct
  misc_feature 1..19: note = SR004505S
  source 1..19: mol_type = other RNA
ttgcctttttacagccaaa

SEQ ID NO: 233 - RNA, 19 nt, synthetic construct
  misc_feature 1..19: note = SR004506S
  source 1..19: mol_type = other RNA
acttttctagacctgtttt

SEQ ID NO: 234 - RNA, 19 nt, synthetic construct
  misc_feature 1..19: note = SR004507S
  source 1..19: mol_type = other RNA
cttttctagacctgtttta

SEQ ID NO: 235 - RNA, 19 nt, synthetic construct
  misc_feature 1..19: note = SR004508S
  source 1..19: mol_type = other RNA
ttttctagacctgttttga

SEQ ID NO: 236 - RNA, 19 nt, synthetic construct
  misc_feature 1..19: note = SR004509S
  source 1..19: mol_type = other RNA
tttctagacctgttttgct

SEQ ID NO: 237 - RNA, 19 nt, synthetic construct
  misc_feature 1..19: note = SR004510S
  source 1..19: mol_type = other RNA
ttctagacctgttttgctt

SEQ ID NO: 238 - RNA, 19 nt, synthetic construct
  misc_feature 1..19: note = SR004511S
  source 1..19: mol_type = other RNA
tctagacctgttttgcttt

SEQ ID NO: 239 - RNA, 19 nt, synthetic construct
  misc_feature 1..19: note = SR004512S
  source 1..19: mol_type = other RNA
ctagacctgttttgctttt

SEQ ID NO: 240 - RNA, 19 nt, synthetic construct
  misc_feature 1..19: note = SR004513S
  source 1..19: mol_type = other RNA
tagacctgttttgctttta

SEQ ID NO: 241 - RNA, 19 nt, synthetic construct
  misc_feature 1..19: note = SR004514S
  source 1..19: mol_type = other RNA
agacctgttttgcttttgt

SEQ ID NO: 242 - RNA, 19 nt, synthetic construct
  misc_feature 1..19: note = SR004515S
  source 1..19: mol_type = other RNA
gacctgttttgcttttgta

SEQ ID NO: 243 - RNA, 19 nt, synthetic construct
  misc_feature 1..19: note = SR004516S
  source 1..19: mol_type = other RNA
acctgttttgcttttgtaa

SEQ ID NO: 244 - RNA, 19 nt, synthetic construct
  misc_feature 1..19: note = SR004517S
  source 1..19: mol_type = other RNA
cctgttttgcttttgtaaa

SEQ ID NO: 245 - RNA, 19 nt, synthetic construct
  misc_feature 1..19: note = SR004518S
  source 1..19: mol_type = other RNA
ctgttttgcttttgtaact

SEQ ID NO: 246 - RNA, 19 nt, synthetic construct
  misc_feature 1..19: note = SR004519S
  source 1..19: mol_type = other RNA
tgttttgcttttgtaactt

SEQ ID NO: 247 - RNA, 19 nt, synthetic construct
  misc_feature 1..19: note = SR004520S
  source 1..19: mol_type = other RNA
gttttgcttttgtaactta

SEQ ID NO: 248 - RNA, 19 nt, synthetic construct
  misc_feature 1..19: note = SR004521S
  source 1..19: mol_type = other RNA
ttttgcttttgtaacttga

SEQ ID NO: 249 - RNA, 19 nt, synthetic construct
  misc_feature 1..19: note = SR004522S
  source 1..19: mol_type = other RNA
tttgcttttgtaacttgaa

SEQ ID NO: 250 - RNA, 19 nt, synthetic construct
  misc_feature 1..19: note = SR004523S
  source 1..19: mol_type = other RNA
ttgcttttgtaacttgaaa

SEQ ID NO: 251 - RNA, 19 nt, synthetic construct
  misc_feature 1..19: note = SR004524S
  source 1..19: mol_type = other RNA
tgcttttgtaacttgaaga

SEQ ID NO: 252 - RNA, 19 nt, synthetic construct
  misc_feature 1..19: note = SR004525S
  source 1..19: mol_type = other RNA
gcttttgtaacttgaagat

SEQ ID NO: 253 - RNA, 19 nt, synthetic construct
  misc_feature 1..19: note = SR004526S
  source 1..19: mol_type = other RNA
cttttgtaacttgaagata

SEQ ID NO: 254 - RNA, 19 nt, synthetic construct
  misc_feature 1..19: note = SR004527S
  source 1..19: mol_type = other RNA
ttttgtaacttgaagatat

SEQ ID NO: 255 - RNA, 19 nt, synthetic construct
  misc_feature 1..19: note = SR004528S
  source 1..19: mol_type = other RNA
tttgtaacttgaagatatt

SEQ ID NO: 256 - RNA, 19 nt, synthetic construct
  misc_feature 1..19: note = SR004529S
  source 1..19: mol_type = other RNA
ttgtaacttgaagatattt

SEQ ID NO: 257 - RNA, 19 nt, synthetic construct
  misc_feature 1..19: note = SR004530S
  source 1..19: mol_type = other RNA
tgtaacttgaagatattta

SEQ ID NO: 258 - RNA, 19 nt, synthetic construct
  misc_feature 1..19: note = SR004531S
  source 1..19: mol_type = other RNA
gtaacttgaagatatttat

SEQ ID NO: 259 - RNA, 19 nt, synthetic construct
  misc_feature 1..19: note = SR004532S
  source 1..19: mol_type = other RNA
taacttgaagatatttatt

SEQ ID NO: 260 - RNA, 19 nt, synthetic construct
  misc_feature 1..19: note = SR004533S
  source 1..19: mol_type = other RNA
aacttgaagatatttatta

SEQ ID NO: 261 - RNA, 19 nt, synthetic construct
  misc_feature 1..19: note = SR004534S
  source 1..19: mol_type = other RNA
acttgaagatatttattct

SEQ ID NO: 262 - RNA, 19 nt, synthetic construct
  misc_feature 1..19: note = SR004535S
  source 1..19: mol_type = other RNA
cttgaagatatttattcta

SEQ ID NO: 263 - RNA, 19 nt, synthetic construct
  misc_feature 1..19: note = SR004536S
  source 1..19: mol_type = other RNA
ttgaagatatttattctga

SEQ ID NO: 264 - RNA, 19 nt, synthetic construct
  misc_feature 1..19: note = SR004537S
  source 1..19: mol_type = other RNA
tgaagatatttattctgga

SEQ ID NO: 265 - RNA, 19 nt, synthetic construct
  misc_feature 1..19: note = SR004538S
  source 1..19: mol_type = other RNA
gaagatatttattctgggt

SEQ ID NO: 266 - RNA, 19 nt, synthetic construct
  misc_feature 1..19: note = SR004539S
  source 1..19: mol_type = other RNA
aagatatttattctgggtt

SEQ ID NO: 267 - RNA, 19 nt, synthetic construct
  misc_feature 1..19: note = SR004540S
  source 1..19: mol_type = other RNA
agatatttattctgggttt

SEQ ID NO: 268 - RNA, 19 nt, synthetic construct
  misc_feature 1..19: note = SR004541S
  source 1..19: mol_type = other RNA
gatatttattctgggtttt

SEQ ID NO: 269 - RNA, 19 nt, synthetic construct
  misc_feature 1..19: note = SR004542S
  source 1..19: mol_type = other RNA
atatttattctgggtttta

SEQ ID NO: 270 - RNA, 19 nt, synthetic construct
  misc_feature 1..19: note = SR004543S
  source 1..19: mol_type = other RNA
tatttattctgggttttgt

SEQ ID NO: 271 - RNA, 19 nt, synthetic construct
  misc_feature 1..19: note = SR004544S
  source 1..19: mol_type = other RNA
atttattctgggttttgta

SEQ ID NO: 272 - RNA, 19 nt, synthetic construct
  misc_feature 1..19: note = SR004545S
  source 1..19: mol_type = other RNA
tttattctgggttttgtaa

SEQ ID NO: 273 - RNA, 19 nt, synthetic construct
  misc_feature 1..19: note = SR004546S
  source 1..19: mol_type = other RNA
ttattctgggttttgtaga

SEQ ID NO: 274 - RNA, 19 nt, synthetic construct
  misc_feature 1..19: note = SR004547S
  source 1..19: mol_type = other RNA
tattctgggttttgtagca

SEQ ID NO: 275 - RNA, 19 nt, synthetic construct
  misc_feature 1..19: note = SR004548S
  source 1..19: mol_type = other RNA
attctgggttttgtagcat

SEQ ID NO: 276 - RNA, 19 nt, synthetic construct
  misc_feature 1..19: note = SR004549S
  source 1..19: mol_type = other RNA
ttctgggttttgtagcatt

SEQ ID NO: 277 - RNA, 19 nt, synthetic construct
  misc_feature 1..19: note = SR004550S
  source 1..19: mol_type = other RNA
tctgggttttgtagcattt

SEQ ID NO: 278 - RNA, 19 nt, synthetic construct
  misc_feature 1..19: note = SR004551S
  source 1..19: mol_type = other RNA
ctgggttttgtagcatttt

SEQ ID NO: 279 - RNA, 19 nt, synthetic construct
  misc_feature 1..19: note = SR004552S
  source 1..19: mol_type = other RNA
tgggttttgtagcattttt

SEQ ID NO: 280 - RNA, 19 nt, synthetic construct
  misc_feature 1..19: note = SR004553S
  source 1..19: mol_type = other RNA
gggttttgtagcattttta

SEQ ID NO: 281 - RNA, 19 nt, synthetic construct
  misc_feature 1..19: note = SR004554S
  source 1..19: mol_type = other RNA
ggttttgtagcatttttat

SEQ ID NO: 282 - RNA, 19 nt, synthetic construct
  misc_feature 1..19: note = SR004555S
  source 1..19: mol_type = other RNA
gttttgtagcatttttatt

SEQ ID NO: 283 - RNA, 19 nt, synthetic construct
  misc_feature 1..19: note = SR004556S
  source 1..19: mol_type = other RNA
ttttgtagcatttttatta

SEQ ID NO: 284 - RNA, 19 nt, synthetic construct
  misc_feature 1..19: note = SR004557S
  source 1..19: mol_type = other RNA
tttgtagcatttttattaa

SEQ ID NO: 285 - RNA, 19 nt, synthetic construct
  misc_feature 1..19: note = SR004558S
  source 1..19: mol_type = other RNA
ttgtagcatttttattaat

SEQ ID NO: 286 - RNA, 19 nt, synthetic construct
  misc_feature 1..19: note = SR004559S
  source 1..19: mol_type = other RNA
tgtagcatttttattaata

SEQ ID NO: 287 - RNA, 19 nt, synthetic construct
  misc_feature 1..19: note = SR004560S
  source 1..19: mol_type = other RNA
gtagcatttttattaatat

SEQ ID NO: 288 - RNA, 19 nt, synthetic construct
  misc_feature 1..19: note = SR004561S
  source 1..19: mol_type = other RNA
tagcatttttattaatata

SEQ ID NO: 289 - RNA, 19 nt, synthetic construct
  misc_feature 1..19: note = SR004562S
  source 1..19: mol_type = other RNA
agcatttttattaatatga

SEQ ID NO: 290 - RNA, 19 nt, synthetic construct
  misc_feature 1..19: note = SR004563S
  source 1..19: mol_type = other RNA
ggtgactttttaaaataaa

SEQ ID NO: 291 - RNA, 19 nt, synthetic construct
  misc_feature 1..19: note = SR004564S
  source 1..19: mol_type = other RNA
gtgactttttaaaataaaa

SEQ ID NO: 292 - RNA, 19 nt, synthetic construct
  misc_feature 1..19: note = SR004565S
  source 1..19: mol_type = other RNA
tgactttttaaaataaaaa

SEQ ID NO: 293 - RNA, 19 nt, synthetic construct
  misc_feature 1..19: note = SR004566S
  source 1..19: mol_type = other RNA
gactttttaaaataaaaat

SEQ ID NO: 294 - RNA, 19 nt, synthetic construct
  misc_feature 1..19: note = SR004567S
  source 1..19: mol_type = other RNA
actttttaaaataaaaaca

SEQ ID NO: 295 - RNA, 19 nt, synthetic construct
  misc_feature 1..19: note = SR004568S
  source 1..19: mol_type = other RNA
ctttttaaaataaaaacaa

SEQ ID NO: 296 - RNA, 19 nt, synthetic construct
  misc_feature 1..19: note = SR004569S
  source 1..19: mol_type = other RNA
tttttaaaataaaaacaaa

SEQ ID NO: 297 - RNA, 19 nt, synthetic construct
  misc_feature 1..19: note = SR004570S
  source 1..19: mol_type = other RNA
ttttaaaataaaaacaaat

SEQ ID NO: 298 - RNA, 19 nt, synthetic construct
  misc_feature 1..19: note = SR004571S
  source 1..19: mol_type = other RNA
tttaaaataaaaacaaaca

SEQ ID NO: 299 - RNA, 21 nt, synthetic construct
  source 1..21: mol_type = other RNA
  misc_feature 1..21: note = SR004440S
  misc_feature 11: note = T is dT
ctagacctgttttgcttttgt

SEQ ID NO: 300 - RNA, 19 nt, synthetic construct
  misc_feature 1..19: note = SR004676S
  source 1..19: mol_type = other RNA
tgttttgcttttgtaactt

SEQ ID NO: 301 - RNA, 19 nt, synthetic construct
  misc_feature 1..19: note = SR004677S
  source 1..19: mol_type = other RNA
gttttgcttttgtaactta

SEQ ID NO: 302 - RNA, 19 nt, synthetic construct
  misc_feature 1..19: note = SR004678S
  source 1..19: mol_type = other RNA
ttttgcttttgtaacttga

SEQ ID NO: 303 - RNA, 19 nt, synthetic construct
  misc_feature 1..19: note = SR004679S
  source 1..19: mol_type = other RNA
tgcttttgtaacttgaaga

SEQ ID NO: 304 - RNA, 19 nt, synthetic construct
  misc_feature 1..19: note = SR004680S
  source 1..19: mol_type = other RNA
gcttttgtaacttgaagat

SEQ ID NO: 305 - RNA, 19 nt, synthetic construct
  misc_feature 1..19: note = SR004681S
  source 1..19: mol_type = other RNA
cttttgtaacttgaagata

SEQ ID NO: 306 - RNA, 19 nt, synthetic construct
  misc_feature 1..19: note = SR004682S
  source 1..19: mol_type = other RNA
ttttgtaacttgaagatat

SEQ ID NO: 307 - RNA, 21 nt, synthetic construct
  source 1..21: mol_type = other RNA
  misc_feature 1..21: note = SR011225S
  misc_feature 11: note = T is dT
ctagacctgttttgcttttgt

SEQ ID NO: 308 - RNA, 21 nt, synthetic construct
  source 1..21: mol_type = other RNA
  misc_feature 1..21: note = SR011239S
  misc_feature 11: note = T is dT
ctagacctgttttgcttttgt

SEQ ID NO: 309 - RNA, 19 nt, synthetic construct
  misc_feature 1..19: note = SR011269S
  source 1..19: mol_type = other RNA
gttttgcttttgtaactta

SEQ ID NO: 310 - RNA, 19 nt, synthetic construct
  misc_feature 1..19: note = SR011272S
  source 1..19: mol_type = other RNA
gttttgcttttgtaactta

SEQ ID NO: 311 - RNA, 19 nt, synthetic construct
  misc_feature 1..19: note = SR011271S
  source 1..19: mol_type = other RNA
tgttttgcttttgtaactt

SEQ ID NO: 312 - RNA, 19 nt, synthetic construct
  misc_feature 1..19: note = SR011273S
  source 1..19: mol_type = other RNA
tgcttttgtaacttgaaga

SEQ ID NO: 313 - RNA, 21 nt, synthetic construct
  misc_feature 1..21: note = SR004572A
  source 1..21: mol_type = other RNA
ttcagcaccaccacgtaggtg

SEQ ID NO: 314 - RNA, 21 nt, synthetic construct
  misc_feature 1..21: note = SR004573A
  source 1..21: mol_type = other RNA
taggagatacacctccaccag

SEQ ID NO: 315 - RNA, 21 nt, synthetic construct
  misc_feature 1..21: note = SR004574A
  source 1..21: mol_type = other RNA
aagtcggtgaccatgaccctg

SEQ ID NO: 316 - RNA, 21 nt, synthetic construct
  misc_feature 1..21: note = SR004575A
  source 1..21: mol_type = other RNA
tttccgaataaactccaggcc

SEQ ID NO: 317 - RNA, 21 nt, synthetic construct
  misc_feature 1..21: note = SR004576A
  source 1..21: mol_type = other RNA
tgtgacacaaagcaggtgctg

SEQ ID NO: 318 - RNA, 21 nt, synthetic construct
  misc_feature 1..21: note = SR004577A
  source 1..21: mol_type = other RNA
tcattgatgacatctttggca

SEQ ID NO: 319 - RNA, 21 nt, synthetic construct
  misc_feature 1..21: note = SR004578A
  source 1..21: mol_type = other RNA
tacagtcctgcaaaacagctg

SEQ ID NO: 320 - RNA, 21 nt, synthetic construct
  misc_feature 1..21: note = SR004579A
  source 1..21: mol_type = other RNA
tgactttgcattccagacctg

SEQ ID NO: 321 - RNA, 21 nt, synthetic construct
  misc_feature 1..21: note = SR004580A
  source 1..21: mol_type = other RNA
ttaaagctcagccccagccct

SEQ ID NO: 322 - RNA, 21 nt, synthetic construct
  misc_feature 1..21: note = SR004581A
  source 1..21: mol_type = other RNA
tttctggctcagttcctgctg

SEQ ID NO: 323 - RNA, 21 nt, synthetic construct
  misc_feature 1..21: note = SR004582A
  source 1..21: mol_type = other RNA
taaatgtctgcttgcttgggt

SEQ ID NO: 324 - RNA, 21 nt, synthetic construct
  misc_feature 1..21: note = SR004583A
  source 1..21: mol_type = other RNA
aaggcaacagagaggacagac

SEQ ID NO: 325 - RNA, 21 nt, synthetic construct
  misc_feature 1..21: note = SR004584A
  source 1..21: mol_type = other RNA
aaaggcaacagagaggacaga

SEQ ID NO: 326 - RNA, 21 nt, synthetic construct
  misc_feature 1..21: note = SR004585A
  source 1..21: mol_type = other RNA
aaaaggcaacagagaggacag

SEQ ID NO: 327 - RNA, 21 nt, synthetic construct
  misc_feature 1..21: note = SR004586A
  source 1..21: mol_type = other RNA
aaaaaggcaacagagaggaca

SEQ ID NO: 328 - RNA, 21 nt, synthetic construct
  misc_feature 1..21: note = SR004587A
  source 1..21: mol_type = other RNA
taaaaaggcaacagagaggac

SEQ ID NO: 329 - RNA, 21 nt, synthetic construct
  misc_feature 1..21: note = SR004588A
  source 1..21: mol_type = other RNA
ataaaaaggcaacagagagga

SEQ ID NO: 330 - RNA, 21 nt, synthetic construct
  misc_feature 1..21: note = SR004589A
  source 1..21: mol_type = other RNA
tgtaaaaaggcaacagagagg

SEQ ID NO: 331 - RNA, 21 nt, synthetic construct
  misc_feature 1..21: note = SR004590A
  source 1..21: mol_type = other RNA
ttgtaaaaaggcaacagagag

SEQ ID NO: 332 - RNA, 21 nt, synthetic construct
  misc_feature 1..21: note = SR004591A
  source 1..21: mol_type = other RNA
tctgtaaaaaggcaacagaga

SEQ ID NO: 333 - RNA, 21 nt, synthetic construct
  misc_feature 1..21: note = SR004592A
  source 1..21: mol_type = other RNA
tgctgtaaaaaggcaacagag

SEQ ID NO: 334 - RNA, 21 nt, synthetic construct
  misc_feature 1..21: note = SR004593A
  source 1..21: mol_type = other RNA
tggctgtaaaaaggcaacaga

SEQ ID NO: 335 - RNA, 21 nt, synthetic construct
  misc_feature 1..21: note = SR004594A
  source 1..21: mol_type = other RNA
ttggctgtaaaaaggcaacag

SEQ ID NO: 336 - RNA, 21 nt, synthetic construct
  misc_feature 1..21: note = SR004595A
  source 1..21: mol_type = other RNA
tttggctgtaaaaaggcaaca

SEQ ID NO: 337 - RNA, 21 nt, synthetic construct
  misc_feature 1..21: note = SR004596A
  source 1..21: mol_type = other RNA
aaaacaggtctagaaaagttg

SEQ ID NO: 338 - RNA, 21 nt, synthetic construct
  misc_feature 1..21: note = SR004597A
  source 1..21: mol_type = other RNA
taaaacaggtctagaaaagtt

SEQ ID NO: 339 - RNA, 21 nt, synthetic construct
  misc_feature 1..21: note = SR004598A
  source 1..21: mol_type = other RNA
tcaaaacaggtctagaaaagt

SEQ ID NO: 340 - RNA, 21 nt, synthetic construct
  misc_feature 1..21: note = SR004599A
  source 1..21: mol_type = other RNA
agcaaaacaggtctagaaaag

SEQ ID NO: 341 - RNA, 21 nt, synthetic construct
  misc_feature 1..21: note = SR004600A
  source 1..21: mol_type = other RNA
aagcaaaacaggtctagaaaa

SEQ ID NO: 342 - RNA, 21 nt, synthetic construct
  misc_feature 1..21: note = SR004601A
  source 1..21: mol_type = other RNA
aaagcaaaacaggtctagaaa

SEQ ID NO: 343 - RNA, 21 nt, synthetic construct
  misc_feature 1..21: note = SR004602A
  source 1..21: mol_type = other RNA
aaaagcaaaacaggtctagaa

SEQ ID NO: 344 - RNA, 21 nt, synthetic construct
  misc_feature 1..21: note = SR004603A
  source 1..21: mol_type = other RNA
taaaagcaaaacaggtctaga

SEQ ID NO: 345 - RNA, 21 nt, synthetic construct
  misc_feature 1..21: note = SR004604A
  source 1..21: mol_type = other RNA
acaaaagcaaaacaggtctag

SEQ ID NO: 346 - RNA, 21 nt, synthetic construct
  misc_feature 1..21: note = SR004605A
  source 1..21: mol_type = other RNA
tacaaaagcaaaacaggtcta

SEQ ID NO: 347 - RNA, 21 nt, synthetic construct
  misc_feature 1..21: note = SR004606A
  source 1..21: mol_type = other RNA
ttacaaaagcaaaacaggtct

SEQ ID NO: 348 - RNA, 21 nt, synthetic construct
  misc_feature 1..21: note = SR004607A
  source 1..21: mol_type = other RNA
tttacaaaagcaaaacaggtc

SEQ ID NO: 349 - RNA, 21 nt, synthetic construct
  misc_feature 1..21: note = SR004608A
  source 1..21: mol_type = other RNA
agttacaaaagcaaaacaggt

SEQ ID NO: 350 - RNA, 21 nt, synthetic construct
  misc_feature 1..21: note = SR004609A
  source 1..21: mol_type = other RNA
aagttacaaaagcaaaacagg

SEQ ID NO: 351 - RNA, 21 nt, synthetic construct
  misc_feature 1..21: note = SR004610A
  source 1..21: mol_type = other RNA
taagttacaaaagcaaaacag

SEQ ID NO: 352 - RNA, 21 nt, synthetic construct
  misc_feature 1..21: note = SR004611A
  source 1..21: mol_type = other RNA
tcaagttacaaaagcaaaaca

SEQ ID NO: 353 - RNA, 21 nt, synthetic construct
  misc_feature 1..21: note = SR004612A
  source 1..21: mol_type = other RNA
ttcaagttacaaaagcaaaac

SEQ ID NO: 354 - RNA, 21 nt, synthetic construct
  misc_feature 1..21: note = SR004613A
  source 1..21: mol_type = other RNA
tttcaagttacaaaagcaaaa

SEQ ID NO: 355 - RNA, 21 nt, synthetic construct
  misc_feature 1..21: note = SR004614A
  source 1..21: mol_type = other RNA
tcttcaagttacaaaagcaaa

SEQ ID NO: 356 - RNA, 21 nt, synthetic construct
  misc_feature 1..21: note = SR004615A
  source 1..21: mol_type = other RNA
atcttcaagttacaaaagcaa

SEQ ID NO: 357 - RNA, 21 nt, synthetic construct
  misc_feature 1..21: note = SR004616A
  source 1..21: mol_type = other RNA
tatcttcaagttacaaaagca

SEQ ID NO: 358 - RNA, 21 nt, synthetic construct
  misc_feature 1..21: note = SR004617A
  source 1..21: mol_type = other RNA
atatcttcaagttacaaaagc

SEQ ID NO: 359 - RNA, 21 nt, synthetic construct
  misc_feature 1..21: note = SR004618A
  source 1..21: mol_type = other RNA
aatatcttcaagttacaaaag

SEQ ID NO: 360 - RNA, 21 nt, synthetic construct
  misc_feature 1..21: note = SR004619A
  source 1..21: mol_type = other RNA
aaatatcttcaagttacaaaa

SEQ ID NO: 361 - RNA, 21 nt, synthetic construct
  misc_feature 1..21: note = SR004620A
  source 1..21: mol_type = other RNA
taaatatcttcaagttacaaa

SEQ ID NO: 362 - RNA, 21 nt, synthetic construct
  misc_feature 1..21: note = SR004621A
  source 1..21: mol_type = other RNA
ataaatatcttcaagttacaa

SEQ ID NO: 363 - RNA, 21 nt, synthetic construct
  misc_feature 1..21: note = SR004622A
  source 1..21: mol_type = other RNA
aataaatatcttcaagttaca

SEQ ID NO: 364 - RNA, 21 nt, synthetic construct
  misc_feature 1..21: note = SR004623A
  source 1..21: mol_type = other RNA
taataaatatcttcaagttac

SEQ ID NO: 365 - RNA, 21 nt, synthetic construct
  misc_feature 1..21: note = SR004624A
  source 1..21: mol_type = other RNA
agaataaatatcttcaagtta

SEQ ID NO: 366 - RNA, 21 nt, synthetic construct
  misc_feature 1..21: note = SR004625A
  source 1..21: mol_type = other RNA
tagaataaatatcttcaagtt

SEQ ID NO: 367 - RNA, 21 nt, synthetic construct
  misc_feature 1..21: note = SR004626A
  source 1..21: mol_type = other RNA
tcagaataaatatcttcaagt

SEQ ID NO: 368 - RNA, 21 nt, synthetic construct
  misc_feature 1..21: note = SR004627A
  source 1..21: mol_type = other RNA
tccagaataaatatcttcaag

SEQ ID NO: 369 - RNA, 21 nt, synthetic construct
  misc_feature 1..21: note = SR004628A
  source 1..21: mol_type = other RNA
acccagaataaatatcttcaa

SEQ ID NO: 370 - RNA, 21 nt, synthetic construct
  misc_feature 1..21: note = SR004629A
  source 1..21: mol_type = other RNA
aacccagaataaatatcttca

SEQ ID NO: 371 - RNA, 21 nt, synthetic construct
  misc_feature 1..21: note = SR004630A
  source 1..21: mol_type = other RNA
aaacccagaataaatatcttc

SEQ ID NO: 372 - RNA, 21 nt, synthetic construct
  misc_feature 1..21: note = SR004631A
  source 1..21: mol_type = other RNA
aaaacccagaataaatatctt

SEQ ID NO: 373 - RNA, 21 nt, synthetic construct
  misc_feature 1..21: note = SR004632A
  source 1..21: mol_type = other RNA
taaaacccagaataaatatct

SEQ ID NO: 374 - RNA, 21 nt, synthetic construct
  misc_feature 1..21: note = SR004633A
  source 1..21: mol_type = other RNA
acaaaacccagaataaatatc

SEQ ID NO: 375 - RNA, 21 nt, synthetic construct
  misc_feature 1..21: note = SR004634A
  source 1..21: mol_type = other RNA
tacaaaacccagaataaatat

SEQ ID NO: 376 - RNA, 21 nt, synthetic construct
  misc_feature 1..21: note = SR004635A
  source 1..21: mol_type = other RNA
ttacaaaacccagaataaata

SEQ ID NO: 377 - RNA, 21 nt, synthetic construct
  misc_feature 1..21: note = SR004636A
  source 1..21: mol_type = other RNA
tctacaaaacccagaataaat

SEQ ID NO: 378 - RNA, 21 nt, synthetic construct
  misc_feature 1..21: note = SR004637A
  source 1..21: mol_type = other RNA
tgctacaaaacccagaataaa

SEQ ID NO: 379 - RNA, 21 nt, synthetic construct
  misc_feature 1..21: note = SR004638A
  source 1..21: mol_type = other RNA
atgctacaaaacccagaataa

SEQ ID NO: 380 - RNA, 21 nt, synthetic construct
  misc_feature 1..21: note = SR004639A
  source 1..21: mol_type = other RNA
aatgctacaaaacccagaata

SEQ ID NO: 381 - RNA, 21 nt, synthetic construct
  misc_feature 1..21: note = SR004640A
  source 1..21: mol_type = other RNA
aaatgctacaaaacccagaat

SEQ ID NO: 382 - RNA, 21 nt, synthetic construct
  misc_feature 1..21: note = SR004641A
  source 1..21: mol_type = other RNA
aaaatgctacaaaacccagaa

SEQ ID NO: 383 - RNA, 21 nt, synthetic construct
  misc_feature 1..21: note = SR004642A
  source 1..21: mol_type = other RNA
aaaaatgctacaaaacccaga

SEQ ID NO: 384 - RNA, 21 nt, synthetic construct
  misc_feature 1..21: note = SR004643A
  source 1..21: mol_type = other RNA
taaaaatgctacaaaacccag

SEQ ID NO: 385 - RNA, 21 nt, synthetic construct
  misc_feature 1..21: note = SR004644A
  source 1..21: mol_type = other RNA
ataaaaatgctacaaaaccca

SEQ ID NO: 386 - RNA, 21 nt, synthetic construct
  misc_feature 1..21: note = SR004645A
  source 1..21: mol_type = other RNA
aataaaaatgctacaaaaccc

SEQ ID NO: 387 - RNA, 21 nt, synthetic construct
  misc_feature 1..21: note = SR004646A
  source 1..21: mol_type = other RNA
taataaaaatgctacaaaacc

SEQ ID NO: 388 - RNA, 21 nt, synthetic construct
  misc_feature 1..21: note = SR004647A
  source 1..21: mol_type = other RNA
ttaataaaaatgctacaaaac

SEQ ID NO: 389 - RNA, 21 nt, synthetic construct
  misc_feature 1..21: note = SR004648A
  source 1..21: mol_type = other RNA
attaataaaaatgctacaaaa

SEQ ID NO: 390 - RNA, 21 nt, synthetic construct
  misc_feature 1..21: note = SR004649A
  source 1..21: mol_type = other RNA
tattaataaaaatgctacaaa

SEQ ID NO: 391 - RNA, 21 nt, synthetic construct
  misc_feature 1..21: note = SR004650A
  source 1..21: mol_type = other RNA
atattaataaaaatgctacaa

SEQ ID NO: 392 - RNA, 21 nt, synthetic construct
  misc_feature 1..21: note = SR004651A
  source 1..21: mol_type = other RNA
tatattaataaaaatgctaca

SEQ ID NO: 393 - RNA, 21 nt, synthetic construct
  misc_feature 1..21: note = SR004652A
  source 1..21: mol_type = other RNA
tcatattaataaaaatgctac

SEQ ID NO: 394 - RNA, 21 nt, synthetic construct
  misc_feature 1..21: note = SR004653A
  source 1..21: mol_type = other RNA
tttattttaaaaagtcaccat

SEQ ID NO: 395 - RNA, 21 nt, synthetic construct
  misc_feature 1..21: note = SR004654A
  source 1..21: mol_type = other RNA
ttttattttaaaaagtcacca

SEQ ID NO: 396 - RNA, 21 nt, synthetic construct
  misc_feature 1..21: note = SR004655A
  source 1..21: mol_type = other RNA
tttttattttaaaaagtcacc

SEQ ID NO: 397 - RNA, 21 nt, synthetic construct
  misc_feature 1..21: note = SR004656A
  source 1..21: mol_type = other RNA
atttttattttaaaaagtcac

SEQ ID NO: 398 - RNA, 21 nt, synthetic construct
  misc_feature 1..21: note = SR004657A
  source 1..21: mol_type = other RNA
tgtttttattttaaaaagtca

SEQ ID NO: 399 - RNA, 21 nt, synthetic construct
  misc_feature 1..21: note = SR004658A
  source 1..21: mol_type = other RNA
ttgtttttattttaaaaagtc

SEQ ID NO: 400 - RNA, 21 nt, synthetic construct
  misc_feature 1..21: note = SR004659A
  source 1..21: mol_type = other RNA
tttgtttttattttaaaaagt

SEQ ID NO: 401 - RNA, 21 nt, synthetic construct
  misc_feature 1..21: note = SR004660A
  source 1..21: mol_type = other RNA
atttgtttttattttaaaaag

SEQ ID NO: 402 - RNA, 21 nt, synthetic construct
  misc_feature 1..21: note = SR004661A
  source 1..21: mol_type = other RNA
tgtttgtttttattttaaaaa

SEQ ID NO: 403 - RNA, 23 nt, synthetic construct
  misc_feature 1..23: note = SR004442A
  source 1..23: mol_type = other RNA
acaaaagcaaaacaggtctagaa

SEQ ID NO: 404 - RNA, 21 nt, synthetic construct
  misc_feature 1..21: note = SR004609A
  source 1..21: mol_type = other RNA
aagttacaaaagcaaaacagg

SEQ ID NO: 405 - RNA, 21 nt, synthetic construct
  misc_feature 1..21: note = SR004610A
  source 1..21: mol_type = other RNA
taagttacaaaagcaaaacag

SEQ ID NO: 406 - RNA, 21 nt, synthetic construct
  misc_feature 1..21: note = SR004611A
  source 1..21: mol_type = other RNA
tcaagttacaaaagcaaaaca

SEQ ID NO: 407 - RNA, 21 nt, synthetic construct
  misc_feature 1..21: note = SR004614A
  source 1..21: mol_type = other RNA
tcttcaagttacaaaagcaaa

SEQ ID NO: 408 - RNA, 21 nt, synthetic construct
  misc_feature 1..21: note = SR004615A
  source 1..21: mol_type = other RNA
atcttcaagttacaaaagcaa

SEQ ID NO: 409 - RNA, 21 nt, synthetic construct
  misc_feature 1..21: note = SR004616A
  source 1..21: mol_type = other RNA
tatcttcaagttacaaaagca

SEQ ID NO: 410 - RNA, 21 nt, synthetic construct
  misc_feature 1..21: note = SR004617A
  source 1..21: mol_type = other RNA
atatcttcaagttacaaaagc

SEQ ID NO: 411 - RNA, 23 nt, synthetic construct
  misc_feature 1..23: note = SR004442A
  source 1..23: mol_type = other RNA
acaaaagcaaaacaggtctagaa

SEQ ID NO: 412 - RNA, 23 nt, synthetic construct
  misc_feature 1..23: note = SR004442A
  source 1..23: mol_type = other RNA
acaaaagcaaaacaggtctagaa

SEQ ID NO: 413 - RNA, 21 nt, synthetic construct
  misc_feature 1..21: note = SR004610A
  source 1..21: mol_type = other RNA
taagttacaaaagcaaaacag

SEQ ID NO: 414 - RNA, 21 nt, synthetic construct
  misc_feature 1..21: note = SR004610A
  source 1..21: mol_type = other RNA
taagttacaaaagcaaaacag

SEQ ID NO: 415 - RNA, 21 nt, synthetic construct
  misc_feature 1..21: note = SR004609A
  source 1..21: mol_type = other RNA
aagttacaaaagcaaaacagg

SEQ ID NO: 416 - RNA, 21 nt, synthetic construct
  misc_feature 1..21: note = SR004614A
  source 1..21: mol_type = other RNA
tcttcaagttacaaaagcaaa

SEQ ID NO: 417 - DNA, 20 bp, synthetic construct
  source 1..20: mol_type = other DNA
  misc_feature 1..20: note = primer
acgtggacatccgcaaagac

SEQ ID NO: 418 - DNA, 20 bp, synthetic construct
  source 1..20: mol_type = other DNA
  misc_feature 1..20: note = primer
tcttcattgtgctgggtgcc

SEQ ID NO: 419 - DNA, 25 bp, synthetic construct
  source 1..25: mol_type = other DNA
  misc_feature 1..25: note = primer
aacacagtgctgtctggcggcacca

SEQ ID NO: 420 - DNA, 20 bp, synthetic construct
  source 1..20: mol_type = other DNA
  misc_feature 1..20: note = primer
agaaacgcagattgggctgg

SEQ ID NO: 421 - DNA, 20 bp, synthetic construct
  source 1..20: mol_type = other DNA
  misc_feature 1..20: note = primer
gccatcactcaccgagcttc

SEQ ID NO: 422 - DNA, 27 bp, synthetic construct
  source 1..27: mol_type = other DNA
  misc_feature 1..27: note = primer
tgaggctgggaaggggaacacagacca

SEQ ID NO: 423 - DNA, 20 bp, synthetic construct
  source 1..20: mol_type = other DNA
  misc_feature 1..20: note = primer
cggcaaattcaacggcacag

SEQ ID NO: 424 - DNA, 20 bp, synthetic construct
  source 1..20: mol_type = other DNA
  misc_feature 1..20: note = primer
ccacgacatactcagcaccg

SEQ ID NO: 425 - DNA, 27 bp, synthetic construct
  source 1..27: mol_type = other DNA
  misc_feature 1..27: note = primer
accatcttccaggagcgagaccccact

SEQ ID NO: 426 - DNA, 20 bp, synthetic construct
  source 1..20: mol_type = other DNA
  misc_feature 1..20: note = primer
agaaacgcagattgggctgg

SEQ ID NO: 427 - DNA, 20 bp, synthetic construct
  source 1..20: mol_type = other DNA
  misc_feature 1..20: note = primer
gccatcactcaccgagcttc

SEQ ID NO: 428 - DNA, 27 bp, synthetic construct
  source 1..27: mol_type = other DNA
  misc_feature 1..27: note = primer
tgaggctgggaaggggaacacagacca

SEQ ID NO: 429 - DNA, 20 bp, synthetic construct
  source 1..20: mol_type = other DNA
  misc_feature 1..20: note = primer
acgtggacatccgcaaagac

SEQ ID NO: 430 - DNA, 20 bp, synthetic construct
  source 1..20: mol_type = other DNA
  misc_feature 1..20: note = primer
tcttcattgtgctgggtgcc

SEQ ID NO: 431 - DNA, 25 bp, synthetic construct
  source 1..25: mol_type = other DNA
  misc_feature 1..25: note = primer
aacacagtgctgtctggcggcacca

SEQ ID NO: 432 - DNA, 20 bp, synthetic construct
  source 1..20: mol_type = other DNA
  misc_feature 1..20: note = primer
agaaacgcagattgggctgg

SEQ ID NO: 433 - DNA, 20 bp, synthetic construct
  source 1..20: mol_type = other DNA
  misc_feature 1..20: note = primer
gccatcactcaccgagcttc

SEQ ID NO: 434 - DNA, 27 bp, synthetic construct
  source 1..27: mol_type = other DNA
  misc_feature 1..27: note = primer
tgaggctgggaaggggaacacagacca

SEQ ID NO: 435 - DNA, 20 bp, synthetic construct
  source 1..20: mol_type = other DNA
  misc_feature 1..20: note = primer
cggcaaattcaacggcacag

SEQ ID NO: 436 - DNA, 20 bp, synthetic construct
  source 1..20: mol_type = other DNA
  misc_feature 1..20: note = primer
ccacgacatactcagcaccg

SEQ ID NO: 437 - DNA, 27 bp, synthetic construct
  source 1..27: mol_type = other DNA
  misc_feature 1..27: note = primer
accatcttccaggagcgagaccccact

SEQ ID NO: 438 - DNA, 20 bp, synthetic construct
  source 1..20: mol_type = other DNA
  misc_feature 1..20: note = primer
agaaacgcagattgggctgg

SEQ ID NO: 439 - DNA, 20 bp, synthetic construct
  source 1..20: mol_type = other DNA
  misc_feature 1..20: note = primer
gccatcactcaccgagcttc

SEQ ID NO: 440 - DNA, 27 bp, synthetic construct
  source 1..27: mol_type = other DNA
  misc_feature 1..27: note = primer
tgaggctgggaaggggaacacagacca